European Patent Specification EP 3 488 239 B1, published March 25, 2026. Title: QUANTITATIVE MASSIVELY PARALLEL PROTEOMICS. Applicant: Verily Life Sciences LLC Peikon, Ian Tong, Gary Liu, Daniel Chu, Ci. The sequence listing filed with the application follows.

SEQUENCE LISTING (1 sequence)

SEQ ID NO: 1 - DNA, 50 bp, Artificial sequence
  Synthetic construct
  misc_feature (23)..(23): n is a, c, g, or t
  misc_feature (31)..(31): n is a, c, g, or t
ggtagaagtactagtacgctgtntcttatanacatctccgagcccacgag